European Patent Specification EP 3 292 205 B1, published August 2, 2023. Title: METHODS AND COMPOSITIONS FOR THE PRODUCTION OF UNREDUCED, NON-RECOMBINED GAMETES AND CLONAL OFFSPRING. Applicant: Albertsen, Marc Bernardes de Asis, Joana Brunner, Arco Chamberlin, Mark Chumak, Nina Fox, Tim Grossniklaus, Ueli Lawit, Shai Pasquer, Frederique Williams, Mark. The sequence listing filed with the application follows.

SEQUENCE LISTING (37 sequences)

SEQ ID NO: 1 - protein, 248 aa, Zea mays
MGTEYPTFADVSGARALLFLADSTPRLAPPSRPPALSEEFYCYSGSSSSYSGASTRSCVSDSAQRGRPVDPLRVLSVVASLRRIDPKVLAEATSALFHTDAEKKRKGVWIEIDSGGDDGQSERSSAVASEGSTVTAAASAGSTATSGRCRGAPRVGCAAGGKGPRRAEVIMQWFSQTQAGPATENDIRAAVGDNSGTSKAIRWLLKQEGGLRRAGNGGALDPYVYMAFTSLGGSPWLAVLQPGPHCCR

SEQ ID NO: 2 - protein, 235 aa, Zea mays
MGTEYPTFADVSGARALLFLADSTPRLAPPSRPPALSEEFYCYSGSSSSYSGASTRSCVSDSAQRGRPVDPLRVLSVVASLRRIDPKVLAEATSALFHTDAEKKRKGVWIEIDSGGDDGQSERSSAVASEGSTVTAAASAGSTATSGRCRGAPRVGCAAGGKGPRRAEVIMQWFSQTQAGPATENDIRAAVGDNSGTSKAIRWLLKQEGGLRRAGNGGALDPYVYMVADRSDEVN

SEQ ID NO: 3 - DNA, 1342 bp, Zea mays
cttttcgaaaatcccccacagaatcccatccccccgggccccggcaaccgctggcgctgcctccagccctccaacaccacgaccgccgggcggctcctcctcctctgccggagagctcggcgggcggcatgggaacagagtatcccaccttcgccgacgtatccggggcccgcgcgctcctcttcctcgccgactccacaccccggctggccccgccttcgcgtcctcccgctctcagcgaggagttctactgctactcgggctcctcgtcctcctactccggcgcgtcgacgaggtcatgcgtctccgactcggcacagcgcggtcgccccgtcgatcccctacgcgtgctctccgtcgtcgcctccctccgccgcatcgaccctaaggtgctagccgaggccacaagcgcgctgttccataccgacgcagagaagaagcggaagggcgtgtggatcgagatcgacagcggtggtgacgacggccagagcgagaggagcagcgccgtggccagcgaggggagcaccgtcacggccgccgcgtccgcgggctccacggccacgtcggggagatgccgcggggctccgcgggtgggttgtgctgctggtggtaaggggccgaggagggcggaggtgatcatgcagtggttttcgcagacgcaagctgggccagcgacggagaacgacatccgcgccgccgtcggcgacaactccggcacgagcaaagcgatacgatggctgttgaagcaggagggcggcttgcggcgtgcaggcaatggtggtgccctggatccgtatgtttatatggcgtttaccagcctaggtggaagtccctggctcgctgtgctgcagcctggtccgcattgctgtcgctgaaagctgcatgagaaaggatgagatggtgtgcgacaaggtacggctccgtggtggagttgcctccggcggggcacccggaacaccttcccggtgcgtgcaagccattgtcgtagcccagagcagcgacgcacctcggctcgttgaaggtaaaccagttcttcaccctgtctccgaacgcgtggaagcagaactcggcgtagtctgcaaacgcctcccttcgattgggcacggcgtgcagctgggtcagactgactgacacatggttgaatcaatttgaaatttggtttctagatgtcgtctagtttgcaattcttacacaatctttgggctaagccagcccaggtactgttcatggagtgccaatgggaggtcataatggtagagatttgcatacggcgcgatacctgacttgtatgtatacatatatataaaggttaaccaggaatctgaatgtttcctgaaagaat

SEQ ID NO: 4 - DNA, 747 bp, Zea mays
atgggaacagagtatcccaccttcgccgacgtatccggggcccgcgcgctcctcttcctcgccgactccacaccccggctggccccgccttcgcgtcctcccgctctcagcgaggagttctactgctactcgggctcctcgtcctcctactccggcgcgtcgacgaggtcatgcgtctccgactcggcacagcgcggtcgccccgtcgatcccctacgcgtgctctccgtcgtcgcctccctccgccgcatcgaccctaaggtgctagccgaggccacaagcgcgctgttccataccgacgcagagaagaagcggaagggcgtgtggatcgagatcgacagcggtggtgacgacggccagagcgagaggagcagcgccgtggccagcgaggggagcaccgtcacggccgccgcgtccgcgggctccacggccacgtcggggagatgccgcggggctccgcgggtgggttgtgctgctggtggtaaggggccgaggagggcggaggtgatcatgcagtggttttcgcagacgcaagctgggccagcgacggagaacgacatccgcgccgccgtcggcgacaactccggcacgagcaaagcgatacgatggctgttgaagcaggagggcggcttgcggcgtgcaggcaatggtggtgccctggatccgtatgtttatatggcgtttaccagcctaggtggaagtccctggctcgctgtgctgcagcctggtccgcattgctgtcgctga

SEQ ID NO: 5 - DNA, 708 bp, Zea mays
atgggaacagagtatcccaccttcgccgacgtatccggggcccgcgcgctcctcttcctcgccgactccacaccccggctggccccgccttcgcgtcctcccgctctcagcgaggagttctactgctactcgggctcctcgtcctcctactccggcgcgtcgacgaggtcatgcgtctccgactcggcacagcgcggtcgccccgtcgatcccctacgcgtgctctccgtcgtcgcctccctccgccgcatcgaccctaaggtgctagccgaggccacaagcgcgctgttccataccgacgcagagaagaagcggaagggcgtgtggatcgagatcgacagcggtggtgacgacggccagagcgagaggagcagcgccgtggccagcgaggggagcaccgtcacggccgccgcgtccgcgggctccacggccacgtcggggagatgccgcggggctccgcgggtgggttgtgctgctggtggtaaggggccgaggagggcggaggtgatcatgcagtggttttcgcagacgcaagctgggccagcgacggagaacgacatccgcgccgccgtcggcgacaactccggcacgagcaaagcgatacgatggctgttgaagcaggagggcggcttgcggcgtgcaggcaatggtggtgccctggatccgtatgtttatatggtcgcagacagatcagatgaagttaactaa

SEQ ID NO: 6 - DNA, 1625 bp, Zea mays
aggaccgataaaacgtcatgtacgctaaatacagcgcacggagacattcgctatgcgcccaataataaccgctaaaccagctggtaaaatataccgggccttcttcgcctctacatctagcggacgagcgaccgctcgctatgcactgttcgaacgtgtgctccgcctcctcctgttccctcccgcgcttgctcggaagctatagcgaccgaccctgactcagacgatcggcgtcgtcgtgatcgtcgcggctacgacggcagagaagcgcgtctggcccgatgtcgcgactgggggtatagatggccatttggcactaacacgatgggtcagcccaggcacggcacgaaaaagcacggtccaggcacgacccggtccggttagtatagtgccagtgtctggcacggcacggctatagtgccgtgcctgggccactatctcgacccgtagtgctggcacaggcacgacacggttacgtttttttattttaaaaataatagtttacatatattaagtataagaattcaacatataacacaataaaactgcagctgcattggttagatagatacgtttaagcctctcatgcactaggttgtgggtttgagcccccacaactacacattttttgctaaattctataatatactcagatgggccatagtgccaccgggccggcccggcacgactagcaggctcacgggccgtgcctgggccgtggcagcggcacgccggcccatctaggcacggcagttttgtagccgggcctggcgggcacgccagcccgtttggccatatataactgggggcgacgacggcaaggcgaaagttggaagagccatggcggagaaaccgaagctagcgacgatgacggcagacgaggagcgcgcttggcccagtctcacgggctcttcctagccgtcgtacagtgctttcgggagcttgtgtcggccacctacaacttcgatttcttggacacgtttggaaagaggtggcgttgtggtggttgcacctctcgtacattgcaatgcacatgttcgacaatatgtctgagacatgaacgatgtctttatgtgtccaaaacgaatttcttttacaaaacgtaagtcagatagttctttagcaaaaacgattagtactgtatattacataatataattattttatttattgcatagttccattttggtaacataggaacgtttttttacaagtgactgatttaaatacaatatatattgtggaatttggtaacactctagttatacaggatcgaatttagagaatgttgctgaagataaaaaagatataaatgacagaatcttttatagaaaactataaaaaaataaaaaatatttatttaaaaataaaatttaaacgatattgctggagaacaaaccaacagtccaacgatagttagacttagactgaaactgcgggcctctttcccggacaattttcaatgtcatgggccggattcgaatctgaattgggcccatcaatttaagaggcgaaacacgggcccgcaccgccgcacgccttcggagtttccgcctttcccccagtcgctcgaaattttaaaatggcgctgctcccctgtcatcctcacggccacgcccccgaaa

SEQ ID NO: 7 - DNA, 4377 bp, Zea mays
cttttcgaaaatcccccacagaatcccatccccccgggccccggcaaccgctggcgctgcctccagccctccaacaccacgaccgccgggcggctcctcctcctctgccggagagctcggcgggcggcatgggaacagagtatcccaccttcgccgacgtatccggggcccgcgcgctcctcttcctcgccgactccacaccccggctggccccgccttcgcgtcctcccgctctcaggtacctgcctcgcgtcatctgctcatcgcgctacggaattgcacttcatcaccgcaatttcacccgaccctccgttgcggcgcgcttctctgcattgcagcgaggagttctactgctactcgggctcctcgtcctcctactccggcgcgtcgacgaggtcatgcgtctccgactcggcacagcgcggtcgccccgtcgatcccctacgcgtgctctccgtcgtcgcctccctccgccgcatcgaccctaaggtgtgcaatcggcgagttcatcgactcgtgatcgtgatcagcacgcggttgcgagaatatctcttctgcgattacgcactgatggctctgctccttggctccaggtgctagccgaggccacaagcgcgctgttccataccgacgcagagaagaagcggaagggcgtgtggatcgagatcgacagcggtggtgacgacggccagagcgagaggagcagcgccgtggccagcgaggggagcaccgtcacggccgccgcgtccgcgggctccacggccacgtcggggagatgccgcggggctccgcgggtgggttgtgctgctggtggtaaggggccgaggagggcggaggtgatcatgcagtggttttcgcagacgcaagctgggccagcgacggagaacgacatccgcgccgccgtcggcgacaactccggcacgagcaaagcgatacgatggtgagcttgactctgcctccaacttccatttgaaaaggttttgcaatggttacctgattacttctgcctgacctgtgtatccgcgtatctgtgtgcttctgctcatgcaaaacttgcaggctgttgaagcaggagggcggcttgcggcgtgcaggcaatggtggtgccctggatccgtatgtttatatggtatgttaaacttgagcggactacttgaattaggatggtagttggaattgcatttttaattccggaacatgtactgcgcagctaagaacttcaaatcagcgcaaaatgtaagaattcctagaactgcaaattaggatttaggaacttgccacaagcacgactaagcaatttaaccatatcttagttttcctgaaatgcattatatagttaaatttctgaataaattttcaggtcgcagacagatcagatgaagttaactaagctttgtttatagaaatagcgatggagatgtttactgtaaggcaattggacaggccaagttatcttctgaagtgtatctataataatttctacatgctgttgtcttaatgacctggtttccccctaccacagataagtataggatagaagttaagttgtcatgttagcacggtgaagataagctcttgaacagaaaaacggcgagatagaatctcaagtataagttcagtatataaagtatagcgatgaagctaccatgatttcgttgttgatttgagctatataccgtgtggtcaaatatatatggtttggctaaatggattatcgaataaaatgagttcaattttcagcttgttgaatgtaacgaagttttaattcgccccttttgttttttttatgccgtttatgttggtgaacttgtgtgtcatttgtctgtgatcccgtcattgtgcttctacttgttctattatggagactcaaggttttcgaagataccaatttattgccttgcaacaattaacgaagctagagatgtcgagccttgagactcaattgtctgcacggttccttaagctaaatctgacatactaagaggatttgcagagtgaacttttgtatgacacgtgaagccagtggtcctcttgtctgcaattctctagctccttttcttggacagcatatgcttgaaccagaaagctgaatccttggggtacctcttcagagtcttgtagtccacgtacaccaagccaaaccgcgaagtgtacccaagcctccactcgaagttgtcaagcagcgaccacgcaaagtacccaatgactctggcaccatcatctattgccttcttgagctcagttatgtagtctctgtaataacggattcttactgtgtcatgcacaccctgagtaatactgacatcaccaggttggtccattcctgcaagagcacaccacttaattaattcaaagcatataccgttctacctggaaatttgaatttcgattcatgagttaccgttttcagcaaggatcattgtaggatttttgtaagtttccttgacatagctgacagccttgttgatgccccacggcacaatgtacagccagtaggagtttgcctacagagctcaaagaaatttacagtaccataatcagaggcaaaccaactttcctgctttcgacgtctgaagacatctagcagtacacttacgtgagcgccaataggaactccatttcgttcgtctgcagaaacatgtgaggatcaacatacgactagatgaggtgacggcagcacaagaaactgcggaattcaagaatttggttcgtggagtcagaaacttacagacaaaaccaacatgccaatcatcctggtagctgactggtgtcaggttccatgtcccagggtccttcatgtagaaagaagtgtagtggttgatgccaacatagtctatagagcctttcaccatcctggcttcttcatcgctgaacaacggtagcctgtctttggcaatctcttgcatcgagtacgggtaccgtccatgtacaatggggtcaaggaacctgtaaggatgttgcagtatcagtttgttcttggcaacgagctgtgttggtttgtttccccaaatataagatatcatcagtttgtgtctagttgcctagtacactatagctaataatgtcactgatacaaagaacctctaataagatcagcaatgacaattgggtccttgtataatcaagtgcatgtgctttcaggcgtttaccagcctaggtggaagtccctggctcgctgtgctgcagcctggtccgcattgctgtcgctgaaaggttcgtaccacacgaaatccaggagaattccaatcttccccttctggtgaagctgttcgtttagtggaaaaggaatacggatcattttctggatgcctgaacactgacattttaattactgaactaaatctgcaccgtgcaattcacacttctggttctgggttcggaggcttgaaatatatagttagcaggtctgcattttatttttacctgatacttgtcgcggtatcgcctgacagcagctgcatgagaaaggatgagatggtgtgcgacaaggtacggctccgtggtggagttgcctccggcggggcacccggaacaccttcccggtgcgtgcaagccattgtcgtagcccagagcagcgacgcacctcggctcgttgaaggtaaaccagttcttcaccctgtctccgaacgcgtggaagcagaactcggcgtagtctgcaaacgcctcccttcgattgggcacggcgtgcagctgggtcagactgactgacacatggttgaatcaatttgaaatttggtttctagatgtcgtctagtttgcaattcttacacaatctttgggctaagccagcccaggtactgttcatggagtgccaatgggaggtcataatggtagagatttgcatacggcgcgatacctgacttgtatgtatacatatatataaaggttaaccaggaatctgaatgtttcctgaaagaatatatctatatctatatacataaataactgcctaactgccatatggtggaaacttaccttgctggagcatgtaatctatgagcctgttgtagtaatccactccttcctggtttaccttgccagttccatctgcgtatattatatatacacacagaactctacctcagaaactccttggacccaagaaaattctacagaatggagcacacctacctgggaaaatcctcgaccaagagatcgaaaatcggtacgcatcaaagcccatgttcttcattatgttcacatcttcctgttcctcgaagaacatccgtcaggcgtcacgaaacaacaaggagcacccaaaaacaagaagaacccaatgcattcagagaacacaccttgtaccgatgatactcgtcgaccgtcacgtcagcggtggcattgttagggatggtcccttgtttttttcattccccggat

SEQ ID NO: 8 - DNA, 654 bp, Brachypodium distachyon
atgggttccgctcccgccgccgcggccttcccgacctactccgacttcgccggcgccggcgcgctgctctccctcgccgactcctcgccctcgccacccctccccaccctcaggtcgtgcgtgtccgactcgatccggcgcggccgccccgtcgaccccctccgcgtgctcgccgtcgtcgcctccctccgccgcatcgaccccaaggtgctggccaaggcgaccagtaagctgtgccggggcgaggaggcgaagaagcggaagggcttgtggatcgagatcagcgacgaggaggaggaggacgacgacgacagcgagaggggcagcgcggtggccagcgaggggagcacgatcaccggcgcggcgtccgccggatccacggccacgtcgggaggatgccgccggcctccgcgggcgagcgggggcggcgagaatctgccgcggagggcggactcgatcatggagtggctatcgcggccgaaggcggcgccggccacggagacggccatccgcgccgccgtcggcgacaacgccgtcaccagcaaggcgctgcgctggcttctgaagcagccgagaggcctgcgccgtacaggcagcggtggtcgtgcagatccatttgagtacatggtcctcgagtactttgatcacgcctga

SEQ ID NO: 9 - protein, 217 aa, Brachypodium distachyon
MGSAPAAAAFPTYSDFAGAGALLSLADSSPSPPLPTLRSCVSDSIRRGRPVDPLRVLAVVASLRRIDPKVLAKATSKLCRGEEAKKRKGLWIEISDEEEEDDDDSERGSAVASEGSTITGAASAGSTATSGGCRRPPRASGGGENLPRRADSIMEWLSRPKAAPATETAIRAAVGDNAVTSKALRWLLKQPRGLRRTGSGGRADPFEYMVLEYFDHA

SEQ ID NO: 10 - DNA, 1359 bp, Brachypodium distachyon
atgggttccgctcccgccgccgcggccttcccgacctactccgacttcgccggcgccggcgcgctgctctccctcgccgactcctcgccctcgccacccctccccaccctcaggtacgtgcggctcctgggttggattattctgcgcgcgcgcacttccgagcgcgagacgtactcaccgctcccccgcgcatacatttgcagcgacgagctctcgtcctactcgggctcctcctcctcctactccgtcacctccggcaggtcgtgcgtgtccgactcgatccggcgcggccgccccgtcgaccccctccgcgtgctcgccgtcgtcgcctccctccgccgcatcgaccccaaggtactgaacaagcagccgctcatctgctaattagcgattcaatttggccgtagtgaataatgggggctcggctcgtttgcgctctaggtgctggccaaggcgaccagtaagctgtgccggggcgaggaggcgaagaagcggaagggcttgtggatcgagatcagcgacgaggaggaggaggacgacgacgacagcgagaggggcagcgcggtggccagcgaggggagcacgatcaccggcgcggcgtccgccggatccacggccacgtcgggaggatgccgccggcctccgcgggcgagcgggggcggcgagaatctgccgcggagggcggactcgatcatggagtggctatcgcggccgaaggcggcgccggccacggagacggccatccgcgccgccgtcggcgacaacgccgtcaccagcaaggcgctgcgctggtgagcacaacgcttcctccaatccaattatcgtctgaagaggttttggaatggttgccctgattgctccttctgtgctttgttcgtgcgtctctctgttcgaaatttgcaggcttctgaagcagccgagaggcctgcgccgtacaggcagcggtggtcgtgcagatccatttgagtacatggtacgtgaaatttgtgccgacagagttcgcattggaatgtgaaatgtcaaattcgaaatatattatgactgtttgaatgataatttctcaaggtagcttaacagaacttgagactggatcagtctgaccagcgtgcaaaattcagttatgagtcagtgaggtgttacttgttagcaattttcagttacccagtagagagcagtggaattttaaagcaatcgttaaacctgataaagtttgtgttagttcaagtgatcacctggcttgtataattatggaaggtctattagttgaatcatgaccactgcaaatttggagcaattatgatgtctaattagtaaatcaatttggtatcccaggtcctcgagtactttgatcacgcctga

SEQ ID NO: 11 - DNA, 1700 bp, Brachypodium distachyon
ttagtacttgccagtggtgtgggagtcaacgccggcgcggcgagcgacgccggtggcgcagcccggggtcaggtcagttggtccggccggcgattgggtttgttcggggaggggattttaccattttggacccgagctaagctgctatggtgggcctttgctgagctgagctgcttgctctctcttgtgaaattccgaaggcgtcgacgaaattttttagttccgaatccaccgtcatggcctctcaaatctcaaaatttagaagttcgatttgtttaccggtttttctcttactaagaagaaaatttacgagttgattagaagcttcaagaccatcctaggcctgtaataaagagagcttttcgatgcacacactttgtatttggtgttcatgactcgtgtgttcttgtttgcttacgtaaaagggaaaatgaatatgaggtcaaacttatttgaacgggcacttccgttttgtagtacactcatttcttatgatgtaagatttgaattatgtttaactgtcgtagcgaggaccatgactcgcaattgtaatcttctgaggatgcaaactatggaaatgtggagtattacattgcataatcatcttcagaatgattggcgtctgaaagtacaccggcattaaccatgagcgaaaatagaaaataacaggagactatataaagtgcatcaacgaaggtggaccgatattgactattgactctccatgtcacctatatcggcaataaaatgacttatataatgtgttgtgtctttagattggtcatgaactttgttggcataaaattcagtgataacaaggcttactcttggctagggagtcaattctcttctctcttctccacgccaacaattttcatatcaaaatcaacatttgttgatactctaatttgcaattgagttcgcattgcgcttttttcaagatgttggatcaaatctttttattttcctctaacatactcccactcgccgccgtctcaaacaatgtggtgccgggaagtttcagtcaaaaaattccatctctaagccttcattagccccatgctcctggtggtattttcaaaggtagatttttaattggaaatggtcaaatggaggagagggagaagagaaatcgacttttgtcgaaaaatcaaagtctccagaattcggccaaaagtgtgagctaagaatcaaccttgttatgccctctcctccatttggccaaaagtgtgagctaagaatcacttacaccatcgaatagagcaagtgatggtaatattgactttactgttgtgtatgcttttaaaacccaaattatgccttctccggcttaccataaaaggcaggtcgaagaagcaaggaaagaagacgatttcattaaacaaatcgagtgttcatcaataaatcggaaacgaataaactgattgatcgcatactgaaacaggatcaaaacacgcaatacacacctcgctttacaaactcatcctggcggccccacatgtcagcctgccctatggacctccgccctcacgctcgaaaattcaaaaaacgggaaaggcaacacaacacggctcgtttaaaatccgagagatcagccgcagcatcccaaactcccttcccaaatccccaaacagaacaaaaatcccaactgcaagagcagcagcctctgctgcctcctctctcccgaccgcaccaccacg

SEQ ID NO: 12 - DNA, 957 bp, Sorghum bicolor
atgggccggattcgaatcttgattcggcccatcaatttaagaggcgaacccggacccgcaccggcgttccggcttcccccagacgctcgaaatttcaaaatggcgctgctcccctgtcagcctcacggccacgccaccgaaacttttcgaaaatcccccacaaaatcccagcggccagctccccgaggccccggcaaccgctgcctccgccaccaccgggcgactgctccacctctgccggagagcgcggcgggcggcatgggagcggagtatcccaccttcgaagaggtctccgcggcccgcgtcctcctcctcctcgccgactccacgcccccaccggccctgccttcgcctcctcccacgctcagcgacgagttcttctgctactcgggctcctcatcctcctactccggcgtgtcggcgaggtcgtgcgtctccgactcggcgcagcgcggccgccccgtcgaccccctccgcgtgctctctgtcgtcgcctccctccgccgcctcgaccctaaggtgctcgttgaggccacaagcgcgctgttccataccgacaaagagaagaagcggaagggcgtgtggatcgagatcgacagcggcgatgacgaggatgaccagagcgagaggagcagcgccgtggccagcgaggggagcaccgtcacggccgccgcgtccgcgggctccacggccacgtcggggagatgccgccaggctccgcgggtgggttgtgctgctggtgggactgggaaggggctgaggagggcggacgtgatcatgcagtggttttcacggccgcaagctgggccagccaccgagaatgacatccgcgccgccgtcggcgacaactccggcacgagcaaggcaatacgctggctgctgaagcaggagggcggcttgcggcgtgcaggcactggtggttccctggatccgtatgtttacatggtcgcagactga

SEQ ID NO: 13 - DNA, 1952 bp, Sorghum bicolor
gccgtggactgcgtggtcttgggggtgactgggtgagtaggctctaacggatgttggacttggaccgaactgcaggcctcttttctgggcaattctcactgccatgggccggattcgaatcttgattcggcccatcaatttaagaggcgaacccggacccgcaccggcgttccggcttcccccagacgctcgaaatttcaaaatggcgctgctcccctgtcagcctcacggccacgccaccgaaacttttcgaaaatcccccacaaaatcccagcggccagctccccgaggccccggcaaccgctgcctccgccaccaccgggcgactgctccacctctgccggagagcgcggcgggcggcatgggagcggagtatcccaccttcgaagaggtctccgcggcccgcgtcctcctcctcctcgccgactccacgcccccaccggccctgccttcgcctcctcccacgctcaggtactttcctcgcctgtctcgcgtcatctgctcatcgcaccaccgaattgcacttcatcatcgcaagttaaccgagcctccgttgcggcgcgcttctccgcattacagcgacgagttcttctgctactcgggctcctcatcctcctactccggcgtgtcggcgaggtcgtgcgtctccgactcggcgcagcgcggccgccccgtcgaccccctccgcgtgctctctgtcgtcgcctccctccgccgcctcgaccctaaggtgtgcaatccggttcctcgattgatgatcagcacgcggttacgagcagcctcctctgcagttacgcactgatggctctgttccttggctccaggtgctcgttgaggccacaagcgcgctgttccataccgacaaagagaagaagcggaagggcgtgtggatcgagatcgacagcggcgatgacgaggatgaccagagcgagaggagcagcgccgtggccagcgaggggagcaccgtcacggccgccgcgtccgcgggctccacggccacgtcggggagatgccgccaggctccgcgggtgggttgtgctgctggtgggactgggaaggggctgaggagggcggacgtgatcatgcagtggttttcacggccgcaagctgggccagccaccgagaatgacatccgcgccgccgtcggcgacaactccggcacgagcaaggcaatacgctggtgagcttgactctgcctctgacttccattttaagcggttttgcagtggttgcctgattgctgcctaacctgtgtatctgcgtgcttcctttcgtgcaaaatttgcaggctgctgaagcaggagggcggcttgcggcgtgcaggcactggtggttccctggatccgtatgtttacatggtatgttaaactcgtgcagactacttgaattaggatggtagttggatttgcattttaaaatccacaatgtgtagtgcacacacagctaagaacttcaaatcagtgaattgaaatgtagaattcccataactgcaaagtaggatttaggaacttgccggacgcacgagaagtatatcttaccttttctgatgtgcattacagttattgactcgcatgatatgtcatgtatactaactttctgaataaattttcaggtcgcagactgatccgatgaagttaactaagttttgtttatagcaatggagatgtttactgtaaggctattgcagacgccaagttatcttctgaaatgtatctagtaatttctacctgctgttgtcttaatggccgggttttgccttcacacagaagtataggatagaagttaagttgtcatgttagcacgatgaagataagctcttggacagaaaaatggcaagatagaatctcatgtataaatttagtatagaaagtacagcaatgaagatagcatgctttcgctgttgatttatgctgagacgatatatcgtataaatttagtatcgaataaaatga

SEQ ID NO: 14 - protein, 318 aa, Sorghum bicolor
MGRIRILIRPINLRGEPGPAPAFRLPPDARNFKMALLPCQPHGHATETFRKSPTKSQRPAPRGPGNRCLRHHRATAPPLPESAAGGMGAEYPTFEEVSAARVLLLLADSTPPPALPSPPPTLSDEFFCYSGSSSSYSGVSARSCVSDSAQRGRPVDPLRVLSVVASLRRLDPKVLVEATSALFHTDKEKKRKGVWIEIDSGDDEDDQSERSSAVASEGSTVTAAASAGSTATSGRCRQAPRVGCAAGGTGKGLRRADVIMQWFSRPQAGPATENDIRAAVGDNSGTSKAIRWLLKQEGGLRRAGTGGSLDPYVYMVAD

SEQ ID NO: 15 - DNA, 1700 bp, Sorghum bicolor
aatctcttcaaccccaagatgcactgaaggcagcttctttggtgcaaactccttcttgtccccatgtccaatggttgccctaggccggtcaatctccaatgacatcaaccgtggctgccggtacccgatagcaacaagatcttggagccaagaagtcatgaaatgcaaatccttttcaccccagaatccctcctctgtcatcgcatagcttagatcaagaatccgctcgaatagtgtcctcttactggatcgccactccattaggaactttatcagcttccctacattgacatggagatccttctcttcatcaaatgtgtgagcacgcacattatctatgcggtgcacagttggtgggtagacaactaggtaccctccaatctcccatagtatcctctgcgcccagtatccgcgtatgacatccgatgccattggactcactgacactggcaatgcaagcccccagaacgccggcgagtggaacaatgtgttaacagagttgactggcgtcatcgtgccctgtggtagcgcaaccttgggtgcatccgcgtcaaaccggaaatcaaatgcctccatctccaatgacttccgggtgaagtagaacactgagtcaacatctggaaggccattacacattccttgctgcatgaattggccaccactgaatatctcagtgtagaactcctcagcatccagttcccctgccttctccagcggcagcccccgtggccagaccgacggctgcccaaagtgcacgaacgggttcacgaccgtccggttaggatcggcatggctgtactgcagcagcacggcgcctccctggcgctggtccagatcgacatcgaagtgactggtgaggttgccgcccaggacggcgttgcgcacgtcggcgtcgtagatgacccgcgccccgcgctgcacggcgaagaggtacgccgcggccttgcgcgccgggccccgggctggaaggaaagcgacggagcggaatccgaggtgatcctggtcggcgagcgtgagcaggacggcgcctgggtgggaccaatccgcgggggtcgcctcgtcggcgaccgcgaggagctgccacccggggaccgcgcgcagcgggcggtgccgcggggcatgcggcgacgcgatgaagacgatccagcgagagccgcggaggtccgggtgcggcgaggagaggaggacggggagcgggggcaccttggaccagagcacggacgggtacgggaggcggcggggcgcgcggtaggcggcggggcagagcgcggagggggaggcgccgccgtagaggaggagcagcaggaacggcgccgtggcaagcgccgcgaggaggacgtagacgacgcgcctagatgcgggtctggaggtagtgggcaaggcgttcggtggcatttgggcgttggaggagaaaaggggctggctcgacgacgccgggtccgccggtgagattcggcacttcggccggcgaggggaccggaagggcggacggcgtggagccgtggactgcgtggtcttgggggtgactgggtgagtaggctctaacggatgttggacttggaccgaactgcaggcctcttttctgggcaattctcactgccatgggccggattcgaatcttgattcggcccatcaatttaagaggcgaacccggacccgcaccggcgttccggcttcccccagacgctcgaaatttcaaa

SEQ ID NO: 16 - protein, 263 aa, Panicum virgatum
LRPTPPKLFENPSTGYTPASNSRRPLLLFCRLVGGMGADYPNFADVSGASALLFLADSSPAPPPPPPALSDEISCHSGSSSYSGASASSCVSDSARRGRPVDPLRVLAVVASLRRINPKVLAEATSTLFHSGAEKKRKGVWIDIDSYYDDADQSERSSAVASEGSTVTAATSVGSTATSGRCRRPPRASDCGGGEKPPRRADVIMQWFSRSQAGPATENDIRAAVGDNSGTSKAIRWLLKQKGGLRRAGTGGPLDPYVYMVAG

SEQ ID NO: 17 - DNA, 792 bp, Panicum virgatum
ctcaggcccacaccaccgaaacttttcgaaaatcccagcacgggctacacccctgcctccaactcccggcgacctctcctcctcttttgccggctcgtcggcggcatgggagcggactaccccaacttcgcggacgtctccggggccagcgccctcctcttcctcgccgactcctcgcccgcaccgcctccgcctcctcccgctctcagcgacgagatctcctgtcactcgggctcctcctcctactccggagcgtcggcgagctcgtgcgtttccgactcggcaaggcgcggccgccccgtcgatcccctccgcgtgctagccgttgtcgcctccctccgccgcatcaaccctaaggtgctcgccgaggccacaagcacgctgttccacagcggggcggagaagaagcggaagggtgtgtggattgatatcgacagctactacgacgacgcggaccagagcgagaggagcagcgcggtggctagtgaggggagcaccgtcacggccgccacgtccgtgggctccacggccacgtcgggtagatgccgccggcctccgcgggcgagtgattgtggtggtggtgagaagccgccgaggagggcagacgtgatcatgcagtggttttcgcggtcgcaagctgggccggccacggagaacgatatccgcgccgcggttggggacaactccgggacaagcaaagcgatacgctggctgctgaagcagaaggggggcttgcggcgagcaggcactggcggccccttggatccatatgtttatatggtcgcaggctga

SEQ ID NO: 18 - DNA, 2009 bp, Panicum virgatum
ctcaggcccacaccaccgaaacttttcgaaaatcccagcacgggctacacccctgcctccaactcccggcgacctctcctcctcttttgccggctcgtcggcggcatgggagcggactaccccaacttcgcggacgtctccggggccagcgccctcctcttcctcgccgactcctcgcccgcaccgcctccgcctcctcccgctctcaggtacgttcctccccttcctctcgtcgtaccgccgaattgcgtgaccgcacgcactccgtcgttgcaatttaatcgaccctccgttgtgctgcgcatctgcacattgcagcgacgagatctcctgtcactcgggctcctcctcctactccggagcgtcggcgagctcgtgcgtttccgactcggcaaggcgcggccgccccgtcgatcccctccgcgtgctagccgttgtcgcctccctccgccgcatcaaccctaaggtgagcaatccgattcctcgattgctgatcagcgcgcgattgcaagccgtctcttccgcagttacgcactgaatactgatggctctgctcgttggctccaggtgctcgccgaggccacaagcacgctgttccacagcggggcggagaagaagcggaagggtgtgtggattgatatcgacagctactacgacgacgcggaccagagcgagaggagcagcgcggtggctagtgaggggagcaccgtcacggccgccacgtccgtgggctccacggccacgtcgggtagatgccgccggcctccgcgggcgagtgattgtggtggtggtgagaagccgccgaggagggcagacgtgatcatgcagtggttttcgcggtcgcaagctgggccggccacggagaacgatatccgcgccgcggttggggacaactccgggacaagcaaagcgatacgctggtgagcaggactttgcctccaacacccattttaagcggttttgaaatggttgcctgattgctgcctgaacatgtgtatctgcttgcttctgttcgtgcgaaatttgcaggctgctgaagcagaaggggggcttgcggcgagcaggcactggcggccccttggatccatatgtttatatggtaagataagattcgtgcaagagtacttaaattaggatggtagttggaattggattttaaattcatatgtgttgtgttgagtgaagattgctagtttgttttagaaattttgaattggatctgtatggacctgggttattgtgcaaattttgagtggagacagtgatcagttagctattcacttcttggaatactatacttcactagtatgaagtggcgcagcataggatgacataactgattcaagtgtacactgatcattcttgactttaatatttctagaaattttactgcaaatttcagagatattgtggtctggtagaaaagttgaaaccctgaatatctttgcattttggttaactgtggagtttgtaaaaatgcttgtaggagactagttgtgagataagagcttttgaattgtgagattcagatactgggtctataaggtcttgtgtcagtgtgcaaagttcggattgaaagagttagcaattagcattttgtagtgacccaatatggaataaacatttgaaaagttaagatgaactgctgaaaatgatttgtgcttatcctgctttacaaagatcttacttgactttatagttctgaaggttctatagattgaattatcagctcttatttcttgaatacttaaattatcagctctgtaccacatcggaaagttgaacacctgaaggccaatgcacatccaggaaggtgaaaccaatgaaatgtataatttataaaagtgatgtggttgtcgcagcatagtgtactgttgcaagctcgaatagcagttccaaccacatcctgagttttttaaattttgcagaatatgtattttatagttattaacccacataatttatcgtgtataataactttttgaatgaaatttcaggtcgcaggctga

SEQ ID NO: 19 - DNA, 1700 bp, Panicum virgatum
cttggggacaaactcctccttgtccccatgtccaattgttgcccttggccggtcaatatccagtgacagcaaccgtggttgccggtacccaatagcaaccagatcttgcagccacgcagccatgaaatgcaaatccttttcaccccagaacccttcctctgtcattgcatagctcaaatcaagaatgcgctcaaacagtgtccgcttactggatcgccactccattaggaactttatcaacctccctatattgacatggatgtccttctcatcatcaaatgggtgagcatgcacattatcgatccggtgtaccgttggtggatagaccactaggtaccctccaatctcccatagtatcctttgcgcccagtatccacgtatgacatctgatgccattggactcactgagactgacaatgcaagcccccagaatgccggtgagtggaacaatgtattaacagagttgatgggtgccatcatgccctgcggcagcgcgaccttaggtgcatacacatcaaactggaaatcgaatgcctccatttctaaagacttccgggtgaagtagaacactgcgtcaatatctggaaggccattgcacatcccctgctgtatgaattgcccaccgctgaatatctcagtgtagaaatcctcagcgtccacctcaccggccttctccagcggcagaccccgcggccagaccgacggctgcccaaagtgcacgaacgggttcacgaccttccggttaggatcggcgtggctgtactgcagcagcacggcgcctccctgccgctggtccagattgacatcgaagtgcttggtgaggttcccacccaggacggcgttgcgcgcgtccgcgtcgtagatgacctgcgccccacgctgcacggcgaagaggtacgccgcggccttgcgcgccggccctcgcgcggggaggaaggcgacggagcggaagccgaggcgggcctggtcggcgagcgtgagcagcacagagcccgggtgggaccagtccgctggggtcgccacgtcggcgacggcgaggagctgccacccggggaccgcccgcagcgggcggtgcttcggggcgtgcggtgacgcggagaagacgatccagcgggaggcgcggagggccgggtgcggcgaggtggggagcgccgggagtgggggaacgcgggaccagaccacggatgggtaggggaggcggcgtggggcgcggaacgaggcggggcagagcgcggtgggggaggcgccgccgtagagaaggaggagaaggaagggcgccgaggcgagcgcggcgaggaggacgtaggcgacgcgcttggaggcgcgcggtggcattttggggagggaaagggtgaggtgacctgatgatgtgccagggcctagggaggtggcggcggagagtcaacgccgccggcccaagcgcgacggccgcggcgcctcgctggtggcgcagccggtgtggtcggcactccggccggcgaggggaccggaacgcggaaggcgtggactgtgtgtggagtaggctgcaacggaaatggctttggaccgaactgcgggcctctttcgatggcacgggccgggttagtctctcgattcagcccattaacatacccacgaatcccaaacccgcacgcctctccgagacgcttgaaaattcaaaatggcgctgctcgcctgtcaaaccctccctacctgtcagc

SEQ ID NO: 20 - protein, 284 aa, Setaria italica
MALLSCETLPVDLTPTPPKLFEIPQQNPSPGNRCLHPPVRRPLLLLCQRGGGMGAEYPTFADVSGARALLFLADSSPAPPPPPPPPALSDEFSCYSGSSSSSSYSGASARSCVSDSARRGRPVDPLRVLSVVASLRRINPKMLAEATGALFHSGAEKKRKGVWIEVDSYEDQSERSSTVASEGSTVTAAASAGSTATSGRCRRPPRASGGGDGGGEKAPRRAEVIMQWFSRSQAGPATENDIRAAVGDNSGTSKAIRWLLKQEGGLRRAGTGGLLDPYVYMVAG

SEQ ID NO: 21 - DNA, 1700 bp, Setaria italica
tgaccatctagcttccgcagcttcactatcttattcttcttttttcgttgacttattcgcaagtgaaaaaactttgtattcttgttaccagcgtaagccacaatattctcgaatggttgatcttttaatatattcatagttagtttactgcatatttggtatttccgatctacattagacagggaggctgcaactatcatctacattagacagcttataatcttttaaacgaggatgaagcgtaattaagaaaacaatataatcattatcgaaattagacagcttataggcttttaaacaaggatgaagcatataagtaagaaaacaacacaaacctcttctgtgagggtttgacagtcgtccctcggttgaagataatgttgcgcattgagtcaatagaatcgcgtacagcaatcacaccaaacacttgcagcggccactgtaagtctgccggactgtttccaactttaaccctgatattataaatctgtagactattggagtggccatcatacacatatcggggcacagatgaatttgagtagtccatggccaggaccattgctgcaggtatttgtcagagatttagattcagaccaattagcatcagcaatggtattcctatactaagatgcatgcattttattttcacaaacatatacatcagcccgcgctagatatacatgctagtagaagtcgctagataggactaagaacacttagaactgaattggcaactgacaaggggcgaaaaatattgatgtataatggagaactcactgatgtcctcgaattccaggccgggattccttgcaatccagtcgtcgcggaacttgagatgatccggggcgtatttgcggtagtacgccaataacttgttgtgcgccttcactcccttttctccagcttcctttgcttgtcatatttttcctcgagttccaccattttcttgcgctttatcagtagcatgatctccataaaaattttcatctcggagcgcttccatcatcgcgctctaattttcttctgctcttcttcctgcttgcgattatcctcctcaactttcttgtgctcttcttcctgctcgcgattatcatcctccttccggtaaaagggagggagcaacccgcgattatcctcctcctccggagtctccttccaaaagagaaggaactcctccgaaagattttccatctcgcacggcgcggacacagctgagttggaggaaaccctagataatgccagcacggcggcaccgctttttatgagaggctgagtggtcgcgtaagcaagggctcgtttggtatggtttacggtagctttagcttcgcaattgtagtagtattgtagtaggtgtagttgaagctgcacggagttcaccagtttcacctccttcacagttcattttaagatttcggtatccgttccagcttcgtgctacagtagcacacacggtgcttaatagtgcgggttactggcgcgtagccgaaacccacctatgcggtgccaaaagggcctaaataggccggactctgaactgtgtggagtaagatgtggaccgaactgcggacctctttcgtgtgcagtaggcctttatccgctcttgatggcatgggccggattaggatctcgattgagcccattaaggcacccaccaatcccaaatccgcacgcctctccaagacgccgaaaaattcaaa

SEQ ID NO: 22 - DNA, 3446 bp, Oryza sativa
atggattcagctcttgccgccgccgccgccaccgccgccgtggcggcgttccccaacttcgccgatgtcgccggcgccgtcgcgctcctcgttctcgccgactcgccgccagcgccgtccccgcctccacctcctcccactgtcaggtactacttccgcgcgcagcactctggttttctccattcggtgttcggcgcgacgaattcaccgccccgtgcggcggcgcctccccgttcattgcagcgacgagctctcgtgctactcgggatcctccgcgtcctactccggcacctcggcgaggtcgtgcgtgtccgactccgcgcagcgcggtcgccccgtcgaccccctccgcgtgctcgccgtcgtcgcctccctccgccgcatcgaccccaaggtaaataatctgatgtgctagatcgcgaacgccaatagtttcatcggtgctaatggctctgctcctcgttgactctaggtgctcgccaaggcgacgaacacgctgtttcagggcgagtcgtcgaagaagaggaagggcgtgtggatccacatcgacgacgatgaggacgagagcgagaggaacagcgctgtggccagcgaggggagcaccgtcacggggaccgcgtctgcaagctccacggccacgtcggggagatcccaccggcctccgcgggcgagtggcggtggcgaccagctgccgcgaagggcggacaagatcatgaagtggttgtcgcggccgggagcggtgccggcaacggagacgaccatccgtgcagccgtcggcgacaatgctggcaccagcaaggcgctgcgcttgtgagtaccacactgctgccaattgcaatttgaaacgcttttgaaatggttgtcatgttaatttcaatttgaagcggttttgaaatggttgccatgttaattccaatctgaagcggttttgaaatggtttccgtgttgctaaattgtttgtgtggaatccgcaggctgctgaagcgtccgggctgcttgcgacgttctggctctggtggccgcaatgatccatatgtttacatggtatgtgaaactcatgcctactgtttgaattgagacgggaatacgaaattcgatgcatgttctgtgctgttgaatgatggtggctcattgtattgtagcttaagagattttcagattggagtagtattaccctttgatagtgtgcaaattttttgaatcgagttagtgagctactgagcttagtaatttccagtggcccagtgggacatacacatttgaagcagttcttaaacctgagttaaatttgcggtagtgctcactgatcactctttagtaccccattctagaagctctatttattgtgttgggagctcagcacaggcaaagttcacagcaacagtgacatgttatgacggccactgcacaggcagacatcacaaaatgtgatgtctcaaatttgtgaattatcagctcttattaactttgcagaatacattcattactatttagctattcccatgatttctcatgagtactattttccttttgatgaattttcaggtcacaggctgacccaatgaagttaactaagttgtgtttatagcaaaagagatggtaactgtaaagctattggagaggccaagtgacttctgagcagtatttagtaatttctactacctgtctgtcttaattactgtttaattttgccttcctgcatataagaagtatagccataggagaaagcaaagttcccatgttagaaagagcttgcagatatatttgtaaagataggctactggatagaaatatagacacacaatcatacacccagagattttatgtcatcgcgctttatattagtgtatgtcgaactggagtaatcaagtataatgagttccattttcagacacttctttttgcaattaactgttatctgaacttctctgtgggaatgaaatctgtgctgttgaataggaattattagatattttgaatagtcccttctgtcagctctttattgtacaaatagcctacggttctgatgaacaaatctgtattgaagttcaatccatttatttctccttctgttgcagaagctagtgaagctaccaatctccacattggttgtttttcacatataactaaagctaaactaacgcgctacgatgagcatacgctagagttagctttgttctgaaatctgacagtggaagcctttgaggctttcacagcttgatccttttgtctgcatactttagttcctcttcttactggagagcatgttcttgaaccagaaagctgagtccttggggtacctctttagcgtcttgtagtccacgtagacgatgccaaaacgggaagtgtacccgagcctccactcgaagttgtcaagcaatgaccaagcaaagtatccaatcactttggcaccatcgtctatcgccttcttgagctcagtgatgtagtttctgtagtatctgattcttactgtatcatgcacaccctgagtgatactgacgttgccaggttggtccatacctgtaagagcacaacattgatcatagtgtaagccttctttaatacttttcattgtcaacaaaactattattcggagaatcagggaccattctgatagaattagtaccattttcagaaaggatcattgtagggtttccatatgtttcctttacataggtcacagccttgttgattccccatggcacaatgtaaagccagtaggagtttgcctgcgtgaattcaatcaattcaactattgaagtgtgatgatttaacttgaaattcaacttttcctaactgttcaacatactactgtacaaatgtacaatacattgactgccacttacttgagctccaatgggcacgccgtttcgttcatctggaaaagacatgagtgcatgagcaactgatccaattaaacagtactacaagaaactgaattatgcatcagaaaatcagaaggatttgggggtggagtattcagaactcacaggcaaacccaacatgccagtcatcctgataactggtcggtgtcaggttccatggcccagggtctttcatgtagaaagaggtgtagtggttgatgccaacataatctattgagtctttcaccatcctggactcctcatcactgaaggttggcatcctgtccttgacgatttcgagcatcgagtatgggtaccgaccatggataatggggtcaaggaacctttaaggagatcatagtgtcagtttgctgatccaaaaaaaagggtactttcagactttcagtttgtggctacactatcacaaaaaatctagactgctactagacctgagcatctgaactctggagtaaataatcgataatttgatcctgaaccagatggtgttttcagatttttaccatccgaggtgaaaatctcttgccctctgtgctgcagccctatcagcattgctgtcactga

SEQ ID NO: 23 - DNA, 1700 bp, Oryza sativa
gccgatcaatctccaatgacatcaaccttggctgccggtaaccaacagagaccagatcttgcagccacgcggacatgaactgcaaatccttctctccccagaacccctcctcagtcatcgcataactcaaatcaagaatacgttcaaagagtgtctgcttatgtgaccgccactccattaggaaatctatcagcctccctacactgacatggatatccttctcatcatcaaacgggtgagcatgcacattatccatgcggtgcacggtcggtgggtagaccactaagtaacccccaatctcccataatatgcgctgcgaccaatacccacgtataacatcagctgccattggactcactgatactggcaatgcaagcccccaaaatgccggtgaatggaacagtgtattaactgagttgattggagccatcatgccctgaggaagtgcgaccttaggcgcatctgcatcaaaccggagatcaaaagcttccatttccgatgatttccgagtgaagtagaacacagcgtcaacatccggtaggccattgcacagcccctgctgtatgaactgcccgccaccgaacacctgagtgtagaattcttccacacccacctccccggctttgtgcagcggcaacccccgcggccacaccgacggctgcccaaagtgcacgtagggattcaccaccgtgcggttgggatccgcatggctgtactgcaagagcacgccgcccccttggcgatggtccagatcgacatcgaagtgcttggtgaggttactgcccaggacggcgttgcgcgcgtccgcgtcgtagatgacgcgcgcgccgcgctgcacggcgaagaggtaggcggcggccttgcgggcgtggccgcgcgcggggaggaaggcaacggagcggaacccgaggcgcgcctggtcggcgagcgtgagcagcgcggcgcccgggtgcgaccagtccgggggcgtggtctcgtcggccacggcgaggagctgccacccggggaccgcgggcagcgggcggtggcgcgggtggtgggccgccgcggcgaagatgatccacctggaggcgcgcagcgacgggagcggcgaggacgggagcaccgggagagggggcacgcgcgaccacgcgacagacgggtactggagccggcgcgacgcaccgccggagcgtgcggcggcgaggcagagcgcggacggggacccgccgccgtagaggaggagcagcaggaacggcgccgccgcgagcgccgcgaggacgacgtaggccacgcggcatctggaactcgccatttttgggcgtagtggtggtggcgagatgggagaggggagaggcgacttggtggagtactactactcctccacttggtagtagtggcgttgctgccgaggtggacagctagtcctcgtcggagtcaatggcctcgcggcggcgccgcgcagcccgcgaggttgtttcgccgccggcgacgaggcccgagaggcgacagagagaggggattttccccattttgggcccaatcatgggcctttatgggccttgatgggccgtgtgtagccgtgcctatcctatgggccgttgctttgctggcttgcacacgtcatcgcgtgctggctttccaacacgctcgaaaattcaaaagttgtctcccttttgatatccccacaaaaatctcgagccccacttgccggcgacgag

SEQ ID NO: 24 - protein, 257 aa, Oryza sativa
MDSALAAAAATAAVAAFPNFADVAGAVALLVLADSPPAPSPPPPPPTVSDELSCYSGSSASYSGTSARSCVSDSAQRGRPVDPLRVLAVVASLRRIDPKVLAKATNTLFQGESSKKRKGVWIHIDDDEDESERNSAVASEGSTVTGTASASSTATSGRSHRPPRASGGGDQLPRRADKIMKWLSRPGAVPATETTIRAAVGDNAGTSKALRLLLKRPGCLRRSGSGGRNDPYVYMIFTIRGENLLPSVLQPYQHCCH

SEQ ID NO: 25 - protein, 229 aa, Oryza sativa
MDSALAAAAATAAVAAFPNFADVAGAVALLVLADSPPAPSPPPPPPTVSDELSCYSGSSASYSGTSARSCVSDSAQRGRPVDPLRVLAVVASLRRIDPKVLAKATNTLFQGESSKKRKGVWIHIDDDEDESERNSAVASEGSTVTGTASAGSTATSGRSHRPPRASGGGDQLPRRADKIMKWLSRPGAVPATETTIRAAVGDNAGTSKALRLLHEASGLLATFWLWWPQ

SEQ ID NO: 26 - DNA, 954 bp, Triticum aestivum
ttttagaagcctattagtcaagtcttaattggtaggcttctaacaaaataaatttggttgagcttctagaataaactgggtaggggtagcttatcccaacttattatagaaaccagcaaaagaactggcacttaaaacgtagttcgaggctaaaattacaagatcacgagaaatcgtgaggacaggtaatcgcctcaatatgattccttatcaacatgttctttaaactgattatttcgtagcttaaaatccatacagatgttcctaaatagtagtaaaggccaggaagtccctattcctaggacaacaacattcctagaatcctcaatcctctcccttccgacctgctgctacaacatgccgaccttacaccctctacacgccaataagaactcatggagcttgggtgccaacgatagtcactagtaccattatacagagttactccctccattcataaatataagatattttactatcttttctgaattagatgtatatagacacgttttagtttttcccgcaaaaaagaagaagacacgttttagtttgtttgttcacttatttcagtccgtatgtagtttatattgaaatattcaaacatcttatatttatgaaccgaggggttacattttaagaaggatacttacaaaaatgataggcaaatgaaaaattatgcaacagaaagagttgccccgaatcaaaatccagtaagatctgcagatatcatcctcgacccgtgcggcctggcgagcggcgaccccgcatgtcagccccccttgaacccaaccgcgccgcacgcctccctacacgggcgctacacactttgaaatttcaaaatggcaccgctactgctaccatcctcccccaaaacttctcaattccccaacaaaatccaactccgccactgcctcctcctctcccaccgccacggcctgcccccttgccggcgac

SEQ ID NO: 27 - protein, 236 aa, Triticum aestivum
MGPAPATASRAAAFPTSADVALAGALLCLADSPPAPLLPTLSDELPSYSGSSSSYSVTSARSCVSDAARRSRPIDPLRVLAVIASLRRVDPKVLVQATSKLFQGELAKRRKGVWIEVINGEEEEGGEESERGSVVASEGSTITGPASSRSTATSGRCRRPPLASGGGDALLRRADSIMKWLSRPKAGPATETAIRAAVGDNAVTSKALRWLLKQKRGLRRAGTGGRPDPYVYMIAG

SEQ ID NO: 28 - DNA, 3220 bp, Triticum aestivum
ggacaacaacattcctagaatcctcaatcctctcccttccgacctgctgctacaacatgccgaccttacaccctctacacgccaataagaactcatggagcttgggtgccaacgatagtcactagtaccattatacagagttactccctccattcataaatataagatattttactatcttttctgaattagatgtatatagacacgttttagtttttcccgcaaaaaagaagaagacacgttttagtttgtttgttcacttatttcagtccgtatgtagtttatattgaaatattcaaacatcttatatttatgaaccgaggggttacattttaagaaggatacttacaaaaatgataggcaaatgaaaaattatgcaacagaaagagttgccccgaatcaaaatccagtaagatctgcagatatcatcctcgacccgtgcggcctggcgagcggcgaccccgcatgtcagccccccttgaacccaaccgcgccgcacgcctccctacacgggcgctacacactttgaaatttcaaaatggcaccgctactgctaccatcctcccccaaaacttctcaattccccaacaaaatccctcaattccccaacaaaatccaactccgccactgcctcctcctctcccaccgccacggcctgcccccttgccggcgacatgggcccggcccccgccaccgcctcccgcgccgcggccttccccacctccgccgacgtcgccctcgccggcgcgctgctctgcctcgccgactccccgcccgcgccgctcctccccaccctcaggtaaccgcgaatccgccgtaccgctaactggttttctgcccgcacccgcttccgcgttccgcgacgggcgctcaccgccgcgtgcgcgtctccgcaattgcagcgacgagctcccctcctactcgggctcctcctcctcctactccgtcacctcggcgaggtcgtgcgtgtccgacgcggcgcgccgcagccgccccatcgaccccctccgcgtgctcgccgtcatcgcctccctccgccgcgtcgaccccaaggtaaccaacctcctcgcctgctagttcgcggtttgtccgtcgtgtctgtcttctgcggcgatgcgctgatcgatggttctggtcggtggctctaggtgctggtgcaggcgaccagcaagctgttccagggcgagctggcgaagaggcggaagggagtgtggatcgaggtcatcaacggcgaggaggaggagggcggggaggagagcgagaggggcagcgtggtggccagcgaggggagcaccatcacgggacccgcgtcctcccggtccacggccacgtcggggaggtgccgccgacctccgctggcgagcggtggtggtgacgctctgctgcggagagcggactcgatcatgaagtggctctcacggccgaaggcggggccggccacagagacggccatccgcgccgccgtcggcgacaacgctgtgaccagcaaggctctgcgctggtgagtgggacacttcctccaatccaactgtcgtctgaagatgttctgaaatttgttgcctaactgcccaatctctgtttgttcgtgcgtctctctgttcggaattcgcaggttgctgaagcagaaaagggggttgcgtcgtgcaggcactggtggccgcccggatccgtatgtgtacatggtacgtgaaatttgtgccacacagtttgcgttggaatgggaatgtcagtttcaaaatatactatgtgtgtttggatgatgattgctcaaggtagctgaaaaaaacttgcaatcagtataactcactgtcactatgcaacctttagatgcagttagggagttgttacttattggagtagtaatttccagttacccagtagagagtaagtggaatctgaaaacagttgttaaatctgattaacttatcctagttccactcacagcctcagttctataattctggaagccccattaattgaaccctgaaccctgcaaattttgtggcaacattgatgtctgacgatcaacttggtagcccaggtccttaagtaattattttgaccacattctgagactttctaacttagctgcatgcatactgtacttaccaattcccaggcttctcatgtgtatactaattgtttctacgaattttcagattgcaggctgaagtggtgaagttaagtaagctgtgttatagcgaaggagttggcacctatatatatctgctggaaaggtcaagttagcttttgaagagtatttagtaatttctagcacctgctgtttaatcggtccagttttgcctagccttcccgcaaataacaaatataggataggaatagatatttacgtgttcgcaatagcttgcaaagcactggtgaaaagctcttggatagaaagataaatggatagtcgtatagatggcagtttcatgattacgaagtcattattcatgtgtgtttagaatcagtataatccttgcaagaagtacgagaaataatcggtactgttggaatcagtataataaaatatgatgggttcagttttggggtactggtttgcagtgaattgctcatttggctttcctctgtgaggtcatatgtatgctgttgaaattgtctcatttgatatgatgatattcaattatcccatgtgcttcagtttacctaaactgatctgcttgtggtgttttgactcttgggaaacaagacttagaagacatgtctttgcttcgcattgtattatatataaggacgggcaaagccacaatctcaatggccttttatttcaagtttcttaaagctaagtccgaggttcatttttggggtactggttacattatgattttattctgaaagctggagcaactgatcctcccggatcttgtttgcaatcctagcctctcttcttctctgagagcatgttcttgaaccacaaggctgagtccttggggtacctcttcagagtattgaagtccacatagacgatgccgaaacgggcagtgtagccgagtctccactcgaagttgtcaagcagagaccaagcaaagtacccaaccactcgtgctccattgtctatcgccttcttgagctcggttatgtagtctctgtagaaccggatccttactgtgtcatgtacaccgtcagcgatgctgacatttcctggctggtccattcctgtcagatcataacattgatcattcgtgcccttgttagtgat

SEQ ID NO: 29 - DNA, 1115 bp, Triticum aestivum
aattccccaacaaaatccaactccgccactgcctcctcctctcccaccgccacggcctgcccccttgccggcgacatgggcccggcccccgccaccgcctcccgcgccgcggccttccccacctccgccgacgtcgccctcgccggcgcgctgctctgcctcgccgactccccgcccgcgccgctcctccccaccctcagcgacgagctcccctcctactcgggctcctcctcctcctactccgtcacctcggcgaggtcgtgcgtgtccgacgcggcgcgccgcagccgccccatcgaccccctccgcgtgctcgccgtcatcgcctccctccgccgcgtcgaccccaaggtgctggtgcaggcgaccagcaagctgttccagggcgagctggcgaagaggcggaagggagtgtggatcgaggtcatcaacggcgaggaggaggagggcggggaggagagcgagaggggcagcgtggtggccagcgaggggagcaccatcacgggacccgcgtcctcccggtccacggccacgtcggggaggtgccgccgacctccgctggcgagcggtggtggtgacgctctgctgcggagagcggactcgatcatgaagtggctctcacggccgaaggcggggccggccacagagacggccatccgcgccgccgtcggcgacaacgctgtgaccagcaaggctctgcgctggttgctgaagcagaaaagggggttgcgtcgtgcaggcactggtggccgcccggatccgtatgtgtacatgattgcaggctgaagtggtgaagttaagtaagctgtgttatagcgaaggagttggcacctatatatatctgctggaaaggtcaagttagcttttgaagagtatttagtaatttctagcacctgctgtttaatcggtccagttttgcctagccttcccgcaaataacaaatataggataggaatagatatttacgtgttcgcaatagcttgcaaagcactggtgaaaagctcttggatagaaagataaatggatagtcgtatagatggcagtttcatgattacgaagtcattattcatgtgtgtttagaatcagtataatccttgcaagaagtacgagaaata

SEQ ID NO: 30 - DNA, 27 bp, Artificial sequence
  oligonucleotide
agaagccaacgccawcgcctcyatttc

SEQ ID NO: 31 - DNA, 51 bp, Artificial sequence
  oligonucleotide
caagcagaagacggcatacgagatagaagccaacgccawcgcctcyatttc

SEQ ID NO: 32 - DNA, 58 bp, Artificial sequence
  oligonucleotide
aatgatacggcgaccaccgagatctacactctttccctacacgacgctcttccgatct

SEQ ID NO: 33 - DNA, 82 bp, Artificial sequence
  oligonucleotide
gtcccccagatttgctaggacaccgccgtacccacaccccggatcagttaatatcgtagacataatggccctccctgccatc

SEQ ID NO: 34 - DNA, 21 bp, Artificial sequence
  oligonucleotide
tataaacatacggatccaggg

SEQ ID NO: 35 - DNA, 68 bp, Artificial sequence
  oligonucleotide
catcatgcatgcagcaggctgtgctgtggacctgatcgagtttcaattgatccaagcaagcaagaggg

SEQ ID NO: 36 - DNA, 21 bp, Artificial sequence
  oligonucleotide
ccctggatgcgtatgtttata

SEQ ID NO: 37 - DNA, 442 bp, Artificial sequence
  oligonucleotide
  misc_feature (402)..(402): n is a, c, g, or t
aattgcagagagagaccagtcgttgatcggtcggagatctccccgaatcgatctcgatcggccggaattttgggggccggccgggaggtggatgatggggggtgattaccatctaggcggcgccgtgttggatgatgtaccaacatatcactataggctactttgggaacctcagatccccttcgggattggaggaaattgagatggaaatgaactaatttcttctctaacccccttcaatcacgaaggggattcgagtttccaaactagccctatatatatcagagctagggagggatattgctgcaacatgcatcacgaggtacagatatataattagggttctgctgcaatgttttgactatagatcgttagtgatctgctgtaattaataataatggngatctcgaagcaattctaaacatcatagtagcaggcccag